European Patent Application EP 4 538 377 A1, published April 16, 2025. Title: A method for producing a heterodimer protein, a dimer protein, a monomer protein, and a screening method for a target-reactive heterodimer protein. Applicant: 国立大学法人山形大学. Application JP. The sequence listing filed with the application follows.

SEQUENCE LISTING (24 sequences)

SEQ ID NO: 1 - protein, 82 aa, Streptococcus pyogenes
DSATHIKFSKRDEDGKELAGATMELRDSSGKTISTWISDGQVKDFYLYPGKYTFVETAAPDGYEVATAITFTVNEQGQVTVN

SEQ ID NO: 2 - protein, 13 aa, Streptococcus pyogenes
AHIVMVDAYKPTK

SEQ ID NO: 3 - protein, 186 aa, Halorhabdus utahensis DSM 12940
CVTGDTLVQAGDGRRRIRELAGETAEAGSIEELPNGRTIRDVDIDVWTMTDDETLTRRPVTAIHEYDAPETLYEVTLSTGEEVTVTPDHPFFIEQASGRVETPAEDLQPGDLVFVPEGSAMATDGGIAQIDTSSDRLGPAESGLGDIGLRTIENVESVPDHDYDSVYDLTVEGTHNFLANGMVVHN

SEQ ID NO: 4 - protein, 61 aa, Halorhabdus utahensis DSM 12940
GIAQIDTSSDRLGPAESGLGDIGLRTIENVESVPDHDYDSVYDLTVEGTHNFLANGMVVHN

SEQ ID NO: 5 - protein, 124 aa, Halorhabdus utahensis DSM 12940
CVTGDTLVQAGDGRRRIRELAGETAEAGSIEELPNGRTIRDVDIDVWTMTDDETLTRRPVTAIHEYDAPETLYEVTLSTGEEVTVTPDHPFFIEQASGRVETPAEDLQPGDLVFVPEGSAMATD

SEQ ID NO: 6 - protein, 40 aa, synthetic construct
  REGION 1..40: note = gp41-1 derived C intein
MMLKKILKIEELDERELIDIEVSGNHLFYANDILTHNSAG

SEQ ID NO: 7 - protein, 91 aa, synthetic construct
  REGION 1..91: note = gp41-1 derived N intein
SGYCLDLKTQVQTPQGMKEISNIQVGDLVLSNTGYNEVLNVFPKSKKKSYKITLEDGKEIICSEEHLFPTQTGEMNISGGLKEGMCLYVKE

SEQ ID NO: 8 - protein, 36 aa, synthetic construct
  REGION 1..36: note = Cfa derived C intein
VKIISRKSLGTQNVYDIGVEKDHNFLLKNGLVASNC

SEQ ID NO: 9 - protein, 101 aa, synthetic construct
  REGION 1..101: note = Cfa N derived N intein
CLSYDTEILTVEYGFLPIGKIVEERIECTVYTVDKNGFVYTQPIAQWHNRGEQEVFEYCLEDGSIIRATKDHKFMTTDGQMLPIDEIFERGLDLKQVDGLP

SEQ ID NO: 10 - protein, 5 aa, synthetic construct
  REGION 1..5: note = linker 1
GGGGS

SEQ ID NO: 11 - protein, 6 aa, synthetic construct
  REGION 1..6: note = linker 2
GGGSGG

SEQ ID NO: 12 - protein, 222 aa, synthetic construct
  REGION 1..222: note = VH-CH domain of OKT3
QVQLVQSGGGVVQPGRSLRLSCKASGYTFTRYTMHWVRQAPGKGLEWIGYINPSRGYTNYNQKVKDRFTISRDNSKNTAFLQMDSLRPEDTGVYFCARYYDDHYSLDYWGQGTPVTVSSASTKGPSVFPLAPSSKSTSGGTAALGCLVKDYFPEPVTVSWNSGALTSGVHTFPAVLQSSGLYSLSSVVTVPSSSLGTQTYICNVNHKPSNTKVDKKVEPKSC

SEQ ID NO: 13 - protein, 346 aa, synthetic construct
  REGION 1..346: note = CD3-Fab-H
MEFGLSWLFLVAILKGVQCQVQLVQSGGGVVQPGRSLRLSCKASGYTFTRYTMHWVRQAPGKGLEWIGYINPSRGYTNYNQKVKDRFTISRDNSKNTAFLQMDSLRPEDTGVYFCARYYDDHYSLDYWGQGTPVTVSSASTKGPSVFPLAPSSKSTSGGTAALGCLVKDYFPEPVTVSWNSGALTSGVHTFPAVLQSSGLYSLSSVVTVPSSSLGTQTYICNVNHKPSNTKVDKKVEPKSCDKTSGYCLDLKTQVQTPQGMKEISNIQVGDLVLSNTGYNEVLNVFPKSKKKSYKITLEDGKEIICSEEHLFPTQTGEMNISGGLKEGMCLYVKEGGSGGHHHHHH

SEQ ID NO: 14 - protein, 110 aa, synthetic construct
  REGION 1..110: note = VL-CL domain of OKT3
DIQMTQSPSSLSASVGDRVTITCSASSSVSYMNWYQQTPGKAPKRWIYDTSKLASGVPSRFSGSGSGTDYTFTISSLQPEDIATYYCQQWSSNPFTFGQGTKLQITRTVA

SEQ ID NO: 15 - protein, 235 aa, synthetic construct
  REGION 1..235: note = CD3-Fab-L
MDFQVQIFSFLLISASVIISRGDIQMTQSPSSLSASVGDRVTITCSASSSVSYMNWYQQTPGKAPKRWIYDTSKLASGVPSRFSGSGSGTDYTFTISSLQPEDIATYYCQQWSSNPFTFGQGTKLQITRTVAAPSVFIFPPSDEQLKSGTASVVCLLNNFYPREAKVQWKVDNALQSGNSQESVTEQDSKDSTYSLSSTLTLSKADYEKHKVYACEVTHQGLSSPVTKSFNRGEC

SEQ ID NO: 16 - protein, 223 aa, synthetic construct
  REGION 1..223: note = VH-CH1 domain of Herceptin
EVQLVESGGGLVQPGGSLRLSCAASGFNIKDTYIHWVRQAPGKGLEWVARIYPTNGYTRYADSVKGRFTISADTSKNTAYLQMNSLRAEDTAVYYCSRWGGDGFYAVDYWGQGTLVTVSSASTKGPSVFPLAPSSKSTSGGTAALGCLVKDYFPEPVTVSWNSGALTSGVHTFPAVLQSSGLYSLSSVVTVPSSSLGTQTYICNVNHKPSNTKVDKKVEPKSC

SEQ ID NO: 17 - protein, 357 aa, synthetic construct
  REGION 1..357: note = Her2-Fab-H
MEFGLSWLFLVAILKGVQCEVQLVESGGGLVQPGGSLRLSCAASGFNIKDTYIHWVRQAPGKGLEWVARIYPTNGYTRYADSVKGRFTISADTSKNTAYLQMNSLRAEDTAVYYCSRWGGDGFYAVDYWGQGTLVTVSSASTKGPSVFPLAPSSKSTSGGTAALGCLVKDYFPEPVTVSWNSGALTSGVHTFPAVLQSSGLYSLSSVVTVPSSSLGTQTYICNVNHKPSNTKVDKKVEPKSCDKTCLSYDTEILTVEYGFLPIGKIVEERIECTVYTVDKNGFVYTQPIAQWHNRGEQEVFEYCLEDGSIIRATKDHKFMTTDGQMLPIDEIFERGLDLKQVDGLPGGSGGHHHHHH

SEQ ID NO: 18 - protein, 106 aa, synthetic construct
  REGION 1..106: note = VL-CL domain of Herceptin
DIQMTQSPSSLSASVGDRVTITCRASQDVNTAVAWYQQKPGKAPKLLIYSASFLYSGVPSRFSGSRSGTDFTLTISSLQPEDFATYYCQQHYTTPPTFGQGTKVEI

SEQ ID NO: 19 - protein, 234 aa, synthetic construct
  REGION 1..234: note = Her2-Fab-L
METPAQLLFLLLLWLPESTGDIQMTQSPSSLSASVGDRVTITCRASQDVNTAVAWYQQKPGKAPKLLIYSASFLYSGVPSRFSGSRSGTDFTLTISSLQPEDFATYYCQQHYTTPPTFGQGTKVEIKRTVAAPSVFIFPPSDEQLKSGTASVVCLLNNFYPREAKVQWKVDNALQSGNSQESVTEQDSKDSTYSLSSTLTLSKADYEKHKVYACEVTHQGLSSPVTKSFNRGEC

SEQ ID NO: 20 - protein, 129 aa, synthetic construct
  REGION 1..129: note = Ia1
QVQLQESGGGLVQAGGSLLLSCAASGRTFSSYAMGWFRQAPGKEREFVAAINWSGGSTSYADSVKGRFTISRDNTKNTVYLQMNSLKPEDTAAFYCAATYNPYSRDHYFPRMTTEYDYWGQGTQVTVSS

SEQ ID NO: 21 - protein, 217 aa, synthetic construct
  REGION 1..217: note = Fc
APELLGGPSVFLFPPKPKDTLMISRTPEVTCVVVDVSHEDPEVKFNWYVDGVEVHNAKTKPREEQYNSTYRVVSVLTVLHQDWLNGKEYKCKVSNKALPAPIEKTISKAKGQPREPQVYTLPPSRDELTKNQVSLTCLVKGFYPSDIAVEWESNGQPENNYKTTPPVLDSDGSFFLYSKLTVDKSRWQQGNVFSCSVMHEALHNHYTQKSLSLSPGK

SEQ ID NO: 22 - protein, 505 aa, synthetic construct
  REGION 1..505: note = SpyCatcher-VHH
MEFGLSWLFLVAILKGVQCQVQLQESGGGLVQAGGSLLLSCAASGRTFSSYAMGWFRQAPGKEREFVAAINWSGGSTSYADSVKGRFTISRDNTKNTVYLQMNSLKPEDTAAFYCAATYNPYSRDHYFPRMTTEYDYWGQGTQVTVSSGGSGGDSATHIKFSKRDEDGKELAGATMELRDSSGKTISTWISDGQVKDFYLYPGKYTFVETAAPDGYEVATAITFTVNEQGQVTVNGGGSGGVKIISRKSLGTQNVYDIGVEKDHNFLLKNGLVASNCFNASYTCPPCPAPELLGGPSVFLFPPKPKDTLMISRTPEVTCVVVDVSHEDPEVKFNWYVDGVEVHNAKTKPREEQYNSTYRVVSVLTVLHQDWLNGKEYKCKVSNKALPAPIEKTISKAKGQPREPQVYTLPPSRDELTKNQVSLTCLVKGFYPSDIAVEWESNGQPENNYKTTPPVLDSDGSFFLYSKLTVDKSRWQQGNVFSCSVMHEALHNHYTQKSLSLSPGK

SEQ ID NO: 23 - protein, 115 aa, synthetic construct [sequence omitted]

SEQ ID NO: 24 - protein, 423 aa, synthetic construct
  REGION 1..423: note = SpyTag-VHH
MEFGLSWLFLVAILKGVQCQVQLVESGGALVQPGGSLRLSCAASGFPVNRYSMRWYRQAPGKEREWVAGMSSAGDRSSYEDSVKGRFTISRDDARNTVYLQMNSLKPEDTAVYYCNVNVGFEYWGQGTQVTVSSGGSGGAHIVMVDAYKPTKGGSGGMMLKKILKIEELDERELIDIEVSGNHLFYANDILTHNSAGASYTCPPCPAPELLGGPSVFLFPPKPKDTLMISRTPEVTCVVVDVSHEDPEVKFNWYVDGVEVHNAKTKPREEQYNSTYRVVSVLTVLHQDWLNGKEYKCKVSNKALPAPIEKTISKAKGQPREPQVYTLPPSRDELTKNQVSLTCLVKGFYPSDIAVEWESNGQPENNYKTTPPVLDSDGSFFLYSKLTVDKSRWQQGNVFSCSVMHEALHNHYTQKSLSLSPGK